European Patent Application EP 4 763 863 A1, published June 24, 2026. Title: 抗BCMA单域抗体及其制备方法与应用. Applicant: 浙江康佰裕生物科技有限公司. Application CN. The sequence listing filed with the application follows.

SEQUENCE LISTING (4 sequences)

SEQ ID NO: 1 - protein, 117 aa, synthetic construct
QLQLVESGGGLVQPGGSLKLSCAASGFTFKDYAMNWYRQAPGKEREWVALISSDGGTTEYEQSVKGRFTISRDNAKNTVYLQMNSVKPEDTAVYRCNKFGAGSYNYWGQGTLVTVSS

SEQ ID NO: 2 - DNA, 351 bp, synthetic construct
  source 1..351: mol_type = other DNA
cagttgcagctcgtggagtcaggtggaggcttggtgcagcctggggggtctctgaaactctcctgtgcagcctctggattcaccttcaaagactatgccatgaactggtaccgtcaggctccagggaaggagcgcgagtgggtcgcacttattagtagtgatggtggtaccacagagtatgagcagtccgtgaaggggcgattcaccatctccagagacaatgccaagaacacggtgtatctgcaaatgaacagcgtgaaacctgaggacacggccgtgtatcgctgtaataagttcggagcaggatcctataactactggggccaggggaccctggtcaccgtctccagc

SEQ ID NO: 3 - DNA, 696 bp, synthetic construct
  source 1..696: mol_type = other DNA
gagcccaaatctgctgacaaaactcacacatgcccaccgtgcccagcacctgaactcctggggggaccgtcagtcttcctcttccccccaaaacccaaggacaccctcatgatctcccggacccccgaggtcacatgcgtggtggtggacgtgagccacgaagaccctgaggtcaagttcaactggtacgtggacggcgtggaggtgcataatgccaagacaaagccgcgggaggagcagtacaacagcacgtaccgtgtggtcagcgtcctcaccgtcctgcaccaggactggctgaatggcaaggagtacaagtgcaaggtctccaacaaagccctcccagcccccatcgagaaaaccatctccaaagccaaagggcagccccgagaaccacaggtgtacaccctgcccccatcccgggaggagatgaccaagaaccaggtcagcctgacctgcctggtcaaaggcttctatcccagcgacatcgccgtggagtgggagagcaatgggcagccggagaacaactacaagaccacgcctcccgtgctggactccgacggctccttcttcctctacagcaagctcaccgtggacaagagcaggtggcagcaggggaacgtcttctcatgctccgtgatgcatgaggctctgcacaaccactacacgcagaagagcctctccctgtctccgggtaaa

SEQ ID NO: 4 - protein, 232 aa, synthetic construct
EPKSADKTHTCPPCPAPELLGGPSVFLFPPKPKDTLMISRTPEVTCVVVDVSHEDPEVKFNWYVDGVEVHNAKTKPREEQYNSTYRVVSVLTVLHQDWLNGKEYKCKVSNKALPAPIEKTISKAKGQPREPQVYTLPPSREEMTKNQVSLTCLVKGFYPSDIAVEWESNGQPENNYKTTPPVLDSDGSFFLYSKLTVDKSRWQQGNVFSCSVMHEALHNHYTQKSLSLSPGK